European Patent Specification EP 3 223 616 B1, published June 7, 2023. Title: Synergistic Bacterial Consortia for Solubilizing and Minerailizing Soil Phosphorus. Applicant: Growcentia LLC Wallenstein, Matthew. Application Not Yet Assigned. The sequence listing filed with the application follows.

SEQUENCE LISTING (4 sequences)

SEQ ID NO: 1 - DNA, 1281 bp, Comamonas testosteroni
  misc_feature (37)..(41): n is a, c, g, t or u
  misc_feature (473)..(473): n is a, c, g, t or u
  misc_feature (691)..(691): n is a, c, g, t or u
  misc_feature (1247)..(1247): n is a, c, g, t or u
catcggaacgtgcctagtagtgggggataactactcnnnnnagtagctaataccgcatgagatctacggatgaaagcaggggaccttcgggccttgtgctactagagcggctgatggcagattaggtagttggtggggtaaaggcttaccaagcctgcgatctgtagctggtctgagaggacgaccagccacactgggactgagacacggcccagactcctacgggaggcagcagtggggaattttggacaatgggcgaaagcctgatccagcaatgccgcgtgcaggatgaaggccctcgggttgtaaactgcttttgtacggaacgaaaagcctggggctaatatccccgggtcatgacggtaccgtaagaataagcaccggctaactacgtgccagcagccgcggtaatacgtagggtgcaagcgttaatcggaattactgggcgtaaagcgtgcgcaggcggttttgtnaagacagtggtgaaatccccgggctcaacctggggaactgccattgtgactgcaaggctagagtgcggcagagggggatggaattccgcgtgtagcagtgaaatgcgtagatatgcggaggaacaccgatggcgaaggcaatcccctgggcctgcactgacgctcatgcacgaaagcgtggggagcaaacaggattagataccctgggtagtccacgnccctaaacgatgtcaactggttgttgggtcttaactgactcagtaacgaagctaacgcgtgaagttgaccgcctggggagtacggccgcaaggttgaaactcaaaggaattgacggggacccgcacaagcggtggatgatgtggtttaattcgatgcaacgcgaaaaaccttacccacctttgacatggcaggaacttaccagagatggtttggtgctcgaaagagaacctgcacacaggtgctgcatggctgtcgtcagctcgtgtcgtgagatgttgggttaagtcccgcaacgagcgcaacccttgccattagttgctacattcagttgagcactctaatgggactgccggtgacaaaccggaggaaggtggggatgacgtcaagtcctcatggcccttataggtggggctacacacgtcatacaatggctggtacaaagggttgccaacccgcgagggggagctaatcccataaagccagtcgtagtccggatcgcagtctgcaactcgactgcgtgaagtcggaatcgctagtaatcgtggatcagaatgncacggtgaatacgttcccgggtcttgtacacacc

SEQ ID NO: 2 - DNA, 1286 bp, Pseudomonas putida
  misc_feature (36)..(40): n is a, c, g, t or u
  misc_feature (1247)..(1247): n is a, c, g, t or u
  misc_feature (1249)..(1250): n is a, c, g, t or u
tgcctaggaatctgcctggtagtgggggacaacgtnnnnnaaggaacgctaataccgcatacgtcctacgggagaaagcaggggaccttcgggccttgcgctatcagatgagcctaggtcggattagctagttggtggggtaatggctcaccaaggcgacgatccgtaactggtctgagaggatgatcagtcacactggaactgagacacggtccagactcctacgggaggcagcagtggggaatattggacaatgggcgaaagcctgatccagccatgccgcgtgtgtgaagaaggtcttcggattgtaaagcactttaagttgggaggaagggcagtaagttaataccttgctgttttgacgttaccgacagaataagcaccggctaactctgtgccagcagccgcggtaatacagagggtgcaagcgttaatcggaattactgggcgtaaagcgcgcgtaggtggttcgttaagttggatgtgaaagccccgggctcaacctgggaactgcatccaaaactggcgagctagagtacggtagagggtggtggaatttcctgtgtagcggtgaaatgcgtagatataggaaggaacaccagtggcgaaggcgaccacctggactgatactgacactgaggtgcgaaagcgtggggagcaaacaggattagataccctggtagtccacgccgtaaacgatgtcaactagccgttggaatccttgagattttagtggcgcagctaacgcattaagtttgaccgcctggggagtacggccgcaaggttaaaactcaaatgaattgacgggggcccgcacaagcggtggagcatgtggtttaattcgaagcaacgcgaagaaaccttaccaggccttgacatgcagagaactttccagagatggattggtgccttcgggaactctgacacaggtgctgcatggctgtcgtcagctcgtgtcgtgagatgttgggttaagtcccgtaacgagcgcaacccttgtccttagttaccagcacgttatggtgggcactctaaggagactgccggtgacaaaccggaggaaggtggggatgacgtcaagtcatcatggcccttacggcctgggctacacacgtgctacaatggtcggtacagagggttgccaagccgcgaggtggagctaatctcacaaaaccgatcgtagtccggatcgcagtctgcaactcgactgcgtgaagtcggaatcgctagtaatcgcgaatcagaangnngcggtgaatacgttcccgggccttgtacacaccgcc

SEQ ID NO: 3 - DNA, 1289 bp, Citrobacter freundii
  misc_feature (36)..(38): n is a, c, g, t or u
  misc_feature (40)..(40): n is a, c, g, t or u
  misc_feature (340)..(341): n is a, c, g, t or u
  misc_feature (893)..(893): n is a, c, g, t or u
  misc_feature (896)..(896): n is a, c, g, t or u
  misc_feature (908)..(912): n is a, c, g, t or u
  misc_feature (927)..(927): n is a, c, g, t or u
  misc_feature (1253)..(1255): n is a, c, g, t or u
  misc_feature (1257)..(1257): n is a, c, g, t or u
agtaatgtctgggaaactgcccgatggagggggatnnntnctggaaacggtagctaataccgcataacgtcgcaagaccaaagagggggaccttcgggcctcttgccatcggatgtgcccagatgggattagctagtaggtggggtaacggctcacctaggcgacgatccctagctggtctgagaggatgaccagccacactggaactgagacacggtccagactcctacgggaggcagcagtggggaatattgcacaatgggcgcaagcctgatgcagccatgccgcgtgtatgaagaaggccttcgggttgtaaagtactttcagcgaggaggaaggnnttgtggttaataaccgcagtgattgacgttactcgcagaagaagcaccggctaactccgtgccagcagccgcggtaatacggagggtgcaagcgttaatcggaattactgggcgtaaagcgcacgcaggcggtctgtcaagtcggatgtgaaatccccgggctcaacctgggaactgcatccgaaactggcaggctagagtcttgtagaggggggtagaattccaggtgtagcggtgaaatgcgtagagatctggaggaataccggtggcgaaggcggcccccctggacaaagactgacgctcaggtgcgaaagcgtggggagcaaacaggattagataccctggtagtccacgccgtaaacgatgtcgacttggaggttgtgcccttgaggcgtggcttccggagctaacgcgttaagtcgaccgcctggggagtacggccgcaaggttaaaactcaaatgaattgacgggggcccgcacaagcggtgggagcatgtggtttaattcgatgcaacgcgaagaaccttacctactcttgacatccagagaanttngcagagatgctnnnnntgccttcgggaactnctgagacaggtgctgcatggctgtcgtcagctcgtgttgtgaaatgttgggttaagtcccgcaacgagcgcaacccttatcctttgttgccagcggttcggccgggaactcaaaggagactgccagtgataaactggaggaaggtggggatgacgtcaagtcatcatggcccttacgagtagggctacacacgtgctacaatggcatatacaaagagaagcgacctcgcgagagcaagcggacctcataaagtatgtcgtagtccggattggagtctgcaactcgactccatgaagtcggaatcgctagtaatcgtggatcagaannncncggtgaatacgttcccgggccttgtacacacc

SEQ ID NO: 4 - DNA, 1296 bp, Enterobacter cloacae
  misc_feature (3)..(3): n is a, c, g, t or u
  misc_feature (9)..(9): n is a, c, g, t or u
  misc_feature (11)..(11): n is a, c, g, t or u
  misc_feature (15)..(15): n is a, c, g, t or u
  misc_feature (19)..(19): n is a, c, g, t or u
  misc_feature (27)..(27): n is a, c, g, t or u
  misc_feature (30)..(30): n is a, c, g, t or u
  misc_feature (37)..(40): n is a, c, g, t or u
  misc_feature (42)..(43): n is a, c, g, t or u
  misc_feature (53)..(53): n is a, c, g, t or u
  misc_feature (55)..(55): n is a, c, g, t or u
  misc_feature (58)..(59): n is a, c, g, t or u
  misc_feature (65)..(65): n is a, c, g, t or u
  misc_feature (68)..(69): n is a, c, g, t or u
  misc_feature (79)..(79): n is a, c, g, t or u
  misc_feature (82)..(82): n is a, c, g, t or u
  misc_feature (86)..(86): n is a, c, g, t or u
  misc_feature (97)..(99): n is a, c, g, t or u
  misc_feature (102)..(102): n is a, c, g, t or u
  misc_feature (105)..(108): n is a, c, g, t or u
  misc_feature (113)..(113): n is a, c, g, t or u
  misc_feature (116)..(116): n is a, c, g, t or u
  misc_feature (120)..(122): n is a, c, g, t or u
  misc_feature (126)..(127): n is a, c, g, t or u
  misc_feature (129)..(129): n is a, c, g, t or u
  misc_feature (141)..(143): n is a, c, g, t or u
  misc_feature (145)..(145): n is a, c, g, t or u
  misc_feature (147)..(147): n is a, c, g, t or u
  misc_feature (150)..(153): n is a, c, g, t or u
  misc_feature (165)..(165): n is a, c, g, t or u
  misc_feature (169)..(169): n is a, c, g, t or u
  misc_feature (172)..(172): n is a, c, g, t or u
  misc_feature (175)..(176): n is a, c, g, t or u
  misc_feature (178)..(179): n is a, c, g, t or u
  misc_feature (182)..(182): n is a, c, g, t or u
  misc_feature (184)..(189): n is a, c, g, t or u
  misc_feature (203)..(204): n is a, c, g, t or u
  misc_feature (212)..(212): n is a, c, g, t or u
  misc_feature (215)..(215): n is a, c, g, t or u
  misc_feature (227)..(228): n is a, c, g, t or u
  misc_feature (235)..(235): n is a, c, g, t or u
  misc_feature (246)..(246): n is a, c, g, t or u
  misc_feature (249)..(249): n is a, c, g, t or u
  misc_feature (251)..(251): n is a, c, g, t or u
  misc_feature (256)..(256): n is a, c, g, t or u
  misc_feature (263)..(263): n is a, c, g, t or u
  misc_feature (274)..(275): n is a, c, g, t or u
  misc_feature (277)..(277): n is a, c, g, t or u
  misc_feature (286)..(286): n is a, c, g, t or u
  misc_feature (288)..(288): n is a, c, g, t or u
  misc_feature (296)..(296): n is a, c, g, t or u
  misc_feature (298)..(299): n is a, c, g, t or u
  misc_feature (301)..(303): n is a, c, g, t or u
  misc_feature (308)..(308): n is a, c, g, t or u
  misc_feature (318)..(318): n is a, c, g, t or u
  misc_feature (320)..(320): n is a, c, g, t or u
  misc_feature (324)..(324): n is a, c, g, t or u
  misc_feature (327)..(327): n is a, c, g, t or u
  misc_feature (330)..(330): n is a, c, g, t or u
  misc_feature (333)..(333): n is a, c, g, t or u
  misc_feature (370)..(370): n is a, c, g, t or u
  misc_feature (386)..(386): n is a, c, g, t or u
  misc_feature (433)..(433): n is a, c, g, t or u
  misc_feature (472)..(472): n is a, c, g, t or u
  misc_feature (496)..(497): n is a, c, g, t or u
  misc_feature (505)..(505): n is a, c, g, t or u
  misc_feature (514)..(514): n is a, c, g, t or u
  misc_feature (842)..(843): n is a, c, g, t or u
  misc_feature (851)..(853): n is a, c, g, t or u
  misc_feature (855)..(855): n is a, c, g, t or u
  misc_feature (970)..(970): n is a, c, g, t or u
  misc_feature (1237)..(1237): n is a, c, g, t or u
  misc_feature (1239)..(1239): n is a, c, g, t or u
  misc_feature (1243)..(1243): n is a, c, g, t or u
  misc_feature (1280)..(1280): n is a, c, g, t or u
  misc_feature (1293)..(1294): n is a, c, g, t or u
ctnataccncntaangtcncaagaccnaanagggggnnnntnnggcctcttgncntcnnatgtgnccnnatgggattanctngtangtggggtaacnnntcnccnnnncgacnatncctnnntggnntnagaggatgaccnnncncnctnnnnctgagacacggnccanacnccnncnngangnnnnnntggggaatattgcnncaatgggngcnagcctgatgcanncatgccncgtgtatgaanaangncttcnggttgtnaagtactttcnncngggaggaangngttgaggntnntnnnctcancaattgacgntncccncanaanaancaccggctaactccgtgccagcagccgcggtaatacngagggtgcaagcgttnatcggaattactgggcgtaaagcgcacgcaggcggtctgtcaagtcngatgtgaaatccccgggctcaacctgggaactgcattcnaaactggcaggctagagtcttgtnnaggggggnagaattccnggtgtagcggtgaaatgcgtagagatctggaggaataccggtggcgaaggcggccccctggacaaagactgacgctcaggtgcgaaagcgtggggagcaaacaggattagataccctggtagtccacgccgtaaacgatgtcgacttggaggttgtgcccttgaggcgtggcttccggagctaacgcgttaagtcgaccgcctggggagtacggccgcaaggttaaaactcaaatgaattgacgggggcccgcacaagcggtggagcatgtggtttaattcgatgcaacgcgaagaaccttacctactcttgacatccagagaacttnncagagatnnntnggtgccttcgggaactctgagacaggtgctgcatggctgtcgtcagctcgtgttgtgaaatgttgggttaagtcccgcaacgagcgcaacccttatcctttgttgccagcggttnggccgggaactcaaaggagactgccagtgataaactggaggaaggtggggatgacgtcaagtcatcatggcccttacgagtagggctacacacgtgctacaatggcgcatacaaagagaagcgacctcgcgagagcaagcggacctcataaagtgcgtcgtagtccggattggagtctgcaactcgactccatgaagtcggaatcgctagtaatcgtagatcagaatgctacggtgaatacgttcccgggccttgtacacaccgccngncacnccatgggagtgggttgcaaaagaagtaggtagcttanccttcgggagggnnct